European Patent Application EP 4 223 777 A1, published August 9, 2023. Title: Anti-CD3 antibody and uses thereof. Applicant: INNOVENT BIOLOGICS(SUZHOU)CO., LTD. The sequence listing filed with the application follows.

SEQUENCE LISTING (126 sequences)

SEQ ID NO: 1 - protein, 10 aa, Artificial
  synthetic
GFTFNTYAMN

SEQ ID NO: 2 - protein, 19 aa, Artificial
  synthetic
RIRSKYNNYATYYADSVKD

SEQ ID NO: 3 - protein, 14 aa, Artificial
  synthetic
HGNFGNSYVSWFAY

SEQ ID NO: 4 - protein, 10 aa, Artificial
  synthetic
GFTFGTYAMN

SEQ ID NO: 5 - protein, 10 aa, Artificial
  synthetic
GFTFNGYAMN

SEQ ID NO: 6 - protein, 10 aa, Artificial
  synthetic
GFTFNTAAMN

SEQ ID NO: 7 - protein, 19 aa, Artificial
  synthetic
RISSKYNNYATYYADSVKD

SEQ ID NO: 8 - protein, 14 aa, Artificial
  synthetic
HGNFGQSYVSWFAY

SEQ ID NO: 9 - protein, 19 aa, Artificial
  synthetic
RIRLKYNNYATYYADSVKD

SEQ ID NO: 10 - protein, 19 aa, Artificial
  synthetic
RIRSKANNYATYYADSVKD

SEQ ID NO: 11 - protein, 19 aa, Artificial
  synthetic
RIRSKYGNYATYYADSVKD

SEQ ID NO: 12 - protein, 19 aa, Artificial
  synthetic
RIRSKYNGYATYYADSVKD

SEQ ID NO: 13 - protein, 14 aa, Artificial
  synthetic
AGNFGQSYVSWFAY

SEQ ID NO: 14 - protein, 14 aa, Artificial
  synthetic
HYNFGQSYVSWFAY

SEQ ID NO: 15 - protein, 14 aa, Artificial
  synthetic
HGGFGQSYVSWFAY

SEQ ID NO: 16 - protein, 14 aa, Artificial
  synthetic
HGNAGQSYVSWFAY

SEQ ID NO: 17 - protein, 14 aa, Artificial
  synthetic
HGNFYQSYVSWFAY

SEQ ID NO: 18 - protein, 14 aa, Artificial
  synthetic
HGNFGGSYVSWFAY

SEQ ID NO: 19 - protein, 14 aa, Artificial
  synthetic
HGNFGQRYVSWFAY

SEQ ID NO: 20 - protein, 14 aa, Artificial
  synthetic
HGNFGQSAVSWFAY

SEQ ID NO: 21 - protein, 14 aa, Artificial
  synthetic
HGNFGQSYASWFAY

SEQ ID NO: 22 - protein, 10 aa, Artificial
  synthetic
GFTFSGSAMN

SEQ ID NO: 23 - protein, 19 aa, Artificial
  synthetic
RISLKYNNYATYYADSVKD

SEQ ID NO: 24 - protein, 19 aa, Artificial
  synthetic
RIRSKAGGYATYYADSVKD

SEQ ID NO: 25 - protein, 14 aa, Artificial
  synthetic
HYGFGQSYVSWFAY

SEQ ID NO: 26 - protein, 14 aa, Artificial
  synthetic
HGNAYQSYVSWFAY

SEQ ID NO: 27 - protein, 14 aa, Artificial
  synthetic
HGNFGGRYVSWFAY

SEQ ID NO: 28 - protein, 14 aa, Artificial
  synthetic
HGNFGQSAASWFAY

SEQ ID NO: 29 - protein, 14 aa, Artificial
  synthetic
RSSTGAVTTSNYAN

SEQ ID NO: 30 - protein, 7 aa, Artificial
  synthetic
GTNKRAP

SEQ ID NO: 31 - protein, 9 aa, Artificial
  synthetic
ALWYSNLWV

SEQ ID NO: 32 - protein, 14 aa, Artificial
  synthetic
GSSTGAVTTSNYAN

SEQ ID NO: 33 - protein, 14 aa, Artificial
  synthetic
RSSTGAVGTSNYAN

SEQ ID NO: 34 - protein, 14 aa, Artificial
  synthetic
RSSTGAVTGSNYAN

SEQ ID NO: 35 - protein, 14 aa, Artificial
  synthetic
RSSTGAVTTRNYAN

SEQ ID NO: 36 - protein, 14 aa, Artificial
  synthetic
RSSTGAVTTSGYAN

SEQ ID NO: 37 - protein, 9 aa, Artificial
  synthetic
ALAYSNLWV

SEQ ID NO: 38 - protein, 9 aa, Artificial
  synthetic
ALWASNLWV

SEQ ID NO: 39 - protein, 9 aa, Artificial
  synthetic
ALWYRNLWV

SEQ ID NO: 40 - protein, 9 aa, Artificial
  synthetic
ALWYSGLWV

SEQ ID NO: 41 - protein, 14 aa, Artificial
  synthetic
RSSTGAVGGSNYAN

SEQ ID NO: 42 - protein, 14 aa, Artificial
  synthetic
RSSTGAVTTRGYAN

SEQ ID NO: 43 - protein, 9 aa, Artificial
  synthetic
ALAASNLWV

SEQ ID NO: 44 - protein, 9 aa, Artificial
  synthetic
ALWYRGLWV

SEQ ID NO: 45 - protein, 7 aa, Artificial
  synthetic
GTNSRAP

SEQ ID NO: 46 - protein, 9 aa, Artificial
  synthetic
ALWYSDLWV

SEQ ID NO: 47 - protein, 125 aa, Artificial
  synthetic
EVQLVESGGGLVQPKGSLKLSCAASGFTFNTYAMNWVRQAPGKGLEWVARIRSKYNNYATYYADSVKDRFTISRDDSQSILYLQMNNLKTEDTAMYYCVRHGNFGNSYVSWFAYWGQGTLVTVSS

SEQ ID NO: 48 - protein, 125 aa, Artificial
  synthetic
EVQLVESGGGLVQPGGSLKLSCAASGFTFNTYAMNWVRQASGKGLEWVGRIRSKYNNYATYYADSVKDRFTISRDDSKNTLYLQMNSLKTEDTAVYYCARHGNFGNSYVSWFAYWGQGTTVTVSS

SEQ ID NO: 49 - protein, 125 aa, Artificial
  synthetic
EVQLVESGGGLVQPGGSLKLSCAASGFTFNTYAMNWVRQASGKGLEWVGRIRSKYNNYATYYADSVKDRFTISRDDSKSTLYLQMNSLKTEDTAVYYCARHGNFGNSYVSWFAYWGQGTTVTVSS

SEQ ID NO: 50 - protein, 125 aa, Artificial
  synthetic
EVQLVESGGGLVQPGGSLKLSCAASGFTFNTYAMNWVRQASGKGLEWVGRIRSKYNNYATYYADSVKDRFTISRDDSKSTLYLQMNSLKTEDTAVYYCARHGNFGQSYVSWFAYWGQGTTVTVSS

SEQ ID NO: 51 - protein, 125 aa, Artificial
  synthetic
EVQLVESGGGLVQPGGSLKLSCAASGFTFNTYAMNWVRQASGKGLEWVARIRSKYNNYATYYADSVKDRFTISRDDSKSTLYLQMNSLKTEDTAVYYCARHGNFGQSYVSWFAYWGQGTTVTVSS

SEQ ID NO: 52 - protein, 125 aa, Artificial
  synthetic
EVQLVESGGGLVQPGGSLKLSCAASGFTFGTYAMNWVRQASGKGLEWVGRIRSKYNNYATYYADSVKDRFTISRDDSKSTLYLQMNSLKTEDTAVYYCARHGNFGQSYVSWFAYWGQGTTVTVSS

SEQ ID NO: 53 - protein, 125 aa, Artificial
  synthetic
EVQLVESGGGLVQPGGSLKLSCAASGFTFNGYAMNWVRQASGKGLEWVGRIRSKYNNYATYYADSVKDRFTISRDDSKSTLYLQMNSLKTEDTAVYYCARHGNFGQSYVSWFAYWGQGTTVTVSS

SEQ ID NO: 54 - protein, 125 aa, Artificial
  synthetic
EVQLVESGGGLVQPGGSLKLSCAASGFTFNTAAMNWVRQASGKGLEWVGRIRSKYNNYATYYADSVKDRFTISRDDSKSTLYLQMNSLKTEDTAVYYCARHGNFGQSYVSWFAYWGQGTTVTVSS

SEQ ID NO: 55 - protein, 125 aa, Artificial
  synthetic
EVQLVESGGGLVQPGGSLKLSCAASGFTFNTYAMNWVRQASGKGLEWVGRISSKYNNYATYYADSVKDRFTISRDDSKSTLYLQMNSLKTEDTAVYYCARHGNFGQSYVSWFAYWGQGTTVTVSS

SEQ ID NO: 56 - protein, 125 aa, Artificial
  synthetic
EVQLVESGGGLVQPGGSLKLSCAASGFTFNTYAMNWVRQASGKGLEWVGRIRLKYNNYATYYADSVKDRFTISRDDSKSTLYLQMNSLKTEDTAVYYCARHGNFGQSYVSWFAYWGQGTTVTVSS

SEQ ID NO: 57 - protein, 125 aa, Artificial
  synthetic
EVQLVESGGGLVQPGGSLKLSCAASGFTFNTYAMNWVRQASGKGLEWVGRIRSKANNYATYYADSVKDRFTISRDDSKSTLYLQMNSLKTEDTAVYYCARHGNFGQSYVSWFAYWGQGTTVTVSS

SEQ ID NO: 58 - protein, 125 aa, Artificial
  synthetic
EVQLVESGGGLVQPGGSLKLSCAASGFTFNTYAMNWVRQASGKGLEWVGRIRSKYGNYATYYADSVKDRFTISRDDSKSTLYLQMNSLKTEDTAVYYCARHGNFGQSYVSWFAYWGQGTTVTVSS

SEQ ID NO: 59 - protein, 125 aa, Artificial
  synthetic
EVQLVESGGGLVQPGGSLKLSCAASGFTFNTYAMNWVRQASGKGLEWVGRIRSKYNGYATYYADSVKDRFTISRDDSKSTLYLQMNSLKTEDTAVYYCARHGNFGQSYVSWFAYWGQGTTVTVSS

SEQ ID NO: 60 - protein, 125 aa, Artificial
  synthetic
EVQLVESGGGLVQPGGSLKLSCAASGFTFNTYAMNWVRQASGKGLEWVGRIRSKYNNYATYYADSVKDRFTISRDDSKSTLYLQMNSLKTEDTAVYYCARAGNFGQSYVSWFAYWGQGTTVTVSS

SEQ ID NO: 61 - protein, 125 aa, Artificial
  synthetic
EVQLVESGGGLVQPGGSLKLSCAASGFTFNTYAMNWVRQASGKGLEWVGRIRSKYNNYATYYADSVKDRFTISRDDSKSTLYLQMNSLKTEDTAVYYCARHYNFGQSYVSWFAYWGQGTTVTVSS

SEQ ID NO: 62 - protein, 125 aa, Artificial
  synthetic
EVQLVESGGGLVQPGGSLKLSCAASGFTFNTYAMNWVRQASGKGLEWVGRIRSKYNNYATYYADSVKDRFTISRDDSKSTLYLQMNSLKTEDTAVYYCARHGGFGQSYVSWFAYWGQGTTVTVSS

SEQ ID NO: 63 - protein, 125 aa, Artificial
  synthetic
EVQLVESGGGLVQPGGSLKLSCAASGFTFNTYAMNWVRQASGKGLEWVGRIRSKYNNYATYYADSVKDRFTISRDDSKSTLYLQMNSLKTEDTAVYYCARHGNAGQSYVSWFAYWGQGTTVTVSS

SEQ ID NO: 64 - protein, 125 aa, Artificial
  synthetic
EVQLVESGGGLVQPGGSLKLSCAASGFTFNTYAMNWVRQASGKGLEWVGRIRSKYNNYATYYADSVKDRFTISRDDSKSTLYLQMNSLKTEDTAVYYCARHGNFYQSYVSWFAYWGQGTTVTVSS

SEQ ID NO: 65 - protein, 125 aa, Artificial
  synthetic
EVQLVESGGGLVQPGGSLKLSCAASGFTFNTYAMNWVRQASGKGLEWVGRIRSKYNNYATYYADSVKDRFTISRDDSKSTLYLQMNSLKTEDTAVYYCARHGNFGGSYVSWFAYWGQGTTVTVSS

SEQ ID NO: 66 - protein, 125 aa, Artificial
  synthetic
EVQLVESGGGLVQPGGSLKLSCAASGFTFNTYAMNWVRQASGKGLEWVGRIRSKYNNYATYYADSVKDRFTISRDDSKSTLYLQMNSLKTEDTAVYYCARHGNFGQRYVSWFAYWGQGTTVTVSS

SEQ ID NO: 67 - protein, 125 aa, Artificial
  synthetic
EVQLVESGGGLVQPGGSLKLSCAASGFTFNTYAMNWVRQASGKGLEWVGRIRSKYNNYATYYADSVKDRFTISRDDSKSTLYLQMNSLKTEDTAVYYCARHGNFGQSAVSWFAYWGQGTTVTVSS

SEQ ID NO: 68 - protein, 125 aa, Artificial
  synthetic
EVQLVESGGGLVQPGGSLKLSCAASGFTFNTYAMNWVRQASGKGLEWVGRIRSKYNNYATYYADSVKDRFTISRDDSKSTLYLQMNSLKTEDTAVYYCARHGNFGQSYASWFAYWGQGTTVTVSS

SEQ ID NO: 69 - protein, 125 aa, Artificial
  synthetic
EVQLVESGGGLVQPGGSLKLSCAASGFTFSGSAMNWVRQASGKGLEWVGRIRSKYNNYATYYADSVKDRFTISRDDSKSTLYLQMNSLKTEDTAVYYCARHGNFGQSYVSWFAYWGQGTTVTVSS

SEQ ID NO: 70 - protein, 125 aa, Artificial
  synthetic
EVQLVESGGGLVQPGGSLKLSCAASGFTFNTYAMNWVRQASGKGLEWVGRISLKYNNYATYYADSVKDRFTISRDDSKSTLYLQMNSLKTEDTAVYYCARHGNFGQSYVSWFAYWGQGTTVTVSS

SEQ ID NO: 71 - protein, 125 aa, Artificial
  synthetic
EVQLVESGGGLVQPGGSLKLSCAASGFTFNTYAMNWVRQASGKGLEWVGRIRSKAGGYATYYADSVKDRFTISRDDSKSTLYLQMNSLKTEDTAVYYCARHGNFGQSYVSWFAYWGQGTTVTVSS

SEQ ID NO: 72 - protein, 125 aa, Artificial
  synthetic
EVQLVESGGGLVQPGGSLKLSCAASGFTFNTYAMNWVRQASGKGLEWVGRIRSKYNNYATYYADSVKDRFTISRDDSKSTLYLQMNSLKTEDTAVYYCARHYGFGQSYVSWFAYWGQGTTVTVSS

SEQ ID NO: 73 - protein, 125 aa, Artificial
  synthetic
EVQLVESGGGLVQPGGSLKLSCAASGFTFNTYAMNWVRQASGKGLEWVGRIRSKYNNYATYYADSVKDRFTISRDDSKSTLYLQMNSLKTEDTAVYYCARHGNAYQSYVSWFAYWGQGTTVTVSS

SEQ ID NO: 74 - protein, 125 aa, Artificial
  synthetic
EVQLVESGGGLVQPGGSLKLSCAASGFTFNTYAMNWVRQASGKGLEWVGRIRSKYNNYATYYADSVKDRFTISRDDSKSTLYLQMNSLKTEDTAVYYCARHGNFGGRYVSWFAYWGQGTTVTVSS

SEQ ID NO: 75 - protein, 125 aa, Artificial
  synthetic
EVQLVESGGGLVQPGGSLKLSCAASGFTFNTYAMNWVRQASGKGLEWVGRIRSKYNNYATYYADSVKDRFTISRDDSKSTLYLQMNSLKTEDTAVYYCARHGNFGQSAASWFAYWGQGTTVTVSS

SEQ ID NO: 76 - protein, 109 aa, Artificial
  synthetic
QAVVTQESALTTSPGETVTLTCRSSTGAVTTSNYANWVQEKPDHLFTGLIGGTNKRAPGVPARFSGSLIGDKAALTITGAQTEDEAIYFCALWYSNLWVFGGGTKLTVL

SEQ ID NO: 77 - protein, 109 aa, Artificial
  synthetic
QAVVTQEPSLTVSPGGTVTLTCRSSTGAVTTSNYANWFQQKPGQAPRTLIYGTNKRAPWTPARFSGSLLGGKAALTLLGAQPEDEAEYYCALWYSNLWVFGQGTKLTVL

SEQ ID NO: 78 - protein, 109 aa, Artificial
  synthetic
QAVVTQEPSLTVSPGGTVTLTCRSSTGAVTTSNYANWVQQKPGQAPRTLIGGTNKRAPGVPARFSGSLLGGKAALTLLGAQPEDEAEYYCALWYSNLWVFGQGTKLTVL

SEQ ID NO: 79 - protein, 109 aa, Artificial
  synthetic
QAVVTQEPSLTVSPGGTVTLTCRSSTGAVTTSNYANWVQQKPGQAPRGLIGGTNKRAPGVPARFSGSLLGGKAALTLLGAQPEDEAEYYCALWYSNLWVFGQGTKLTVL

SEQ ID NO: 80 - protein, 109 aa, Artificial
  synthetic
QAVVTQEPSLTVSPGGTVTLTCRSSTGAVTTSNYANWVQQKPGQAPRGLIGGTNKRAPGVPARFSGSLLGDKAALTLLGAQPEDEAEYYCALWYSNLWVFGQGTKLTVL

SEQ ID NO: 81 - protein, 110 aa, Artificial
  synthetic
EIVMTQSPATLSVSPGERATLSCRSSTGAVTTSNYANWYQQKPGQAPRLLIYGTNKRAPGIPARFSGSGSGTEFTLTISSLQSEDFAVYYCALWYSNLWVFGQGTKLTVL

SEQ ID NO: 82 - protein, 110 aa, Artificial
  synthetic
EIVMTQSPATLSVSPGERATLSCRSSTGAVTTSNYANWVQQKPGQAPRLLIGGTNKRAPGVPARFSGSGSGTEFTLTISSLQSEDFAVYYCALWYSNLWVFGQGTKLTVL

SEQ ID NO: 83 - protein, 110 aa, Artificial
  synthetic
EIVMTQSPATLSVSPGERATLSCRSSTGAVTTSNYANWVQQKPGQAPRGLIGGTNKRAPGVPARFSGSGSGTEFTLTISSLQSEDFAVYYCALWYSNLWVFGQGTKLTVL

SEQ ID NO: 84 - protein, 110 aa, Artificial
  synthetic
EIVMTQSPATLSVSPGERATLSCRSSTGAVTTSNYANWVQQKPGQAPRGLIGGTNKRAPGVPARFSGSGSGDEFTLTISSLQSEDFAVYYCALWYSNLWVFGQGTKLTVL

SEQ ID NO: 85 - protein, 109 aa, Artificial
  synthetic
QAVVTQEPSLTVSPGGTVTLTCGSSTGAVTTSNYANWVQQKPGQAPRGLIGGTNKRAPGVPARFSGSLLGDKAALTLLGAQPEDEAEYYCALWYSNLWVFGQGTKLTVL

SEQ ID NO: 86 - protein, 109 aa, Artificial
  synthetic
QAVVTQEPSLTVSPGGTVTLTCRSSTGAVGTSNYANWVQQKPGQAPRGLIGGTNKRAPGVPARFSGSLLGDKAALTLLGAQPEDEAEYYCALWYSNLWVFGQGTKLTVL

SEQ ID NO: 87 - protein, 109 aa, Artificial
  synthetic
QAVVTQEPSLTVSPGGTVTLTCRSSTGAVTGSNYANWVQQKPGQAPRGLIGGTNKRAPGVPARFSGSLLGDKAALTLLGAQPEDEAEYYCALWYSNLWVFGQGTKLTVL

SEQ ID NO: 88 - protein, 109 aa, Artificial
  synthetic
QAVVTQEPSLTVSPGGTVTLTCRSSTGAVTTRNYANWVQQKPGQAPRGLIGGTNKRAPGVPARFSGSLLGDKAALTLLGAQPEDEAEYYCALWYSNLWVFGQGTKLTVL

SEQ ID NO: 89 - protein, 109 aa, Artificial
  synthetic
QAVVTQEPSLTVSPGGTVTLTCRSSTGAVTTSGYANWVQQKPGQAPRGLIGGTNKRAPGVPARFSGSLLGDKAALTLLGAQPEDEAEYYCALWYSNLWVFGQGTKLTVL

SEQ ID NO: 90 - protein, 109 aa, Artificial
  synthetic
QAVVTQEPSLTVSPGGTVTLTCRSSTGAVTTSNYANWVQQKPGQAPRGLIGGTNKRAPGVPARFSGSLLGDKAALTLLGAQPEDEAEYYCALAYSNLWVFGQGTKLTVL

SEQ ID NO: 91 - protein, 109 aa, Artificial
  synthetic
QAVVTQEPSLTVSPGGTVTLTCRSSTGAVTTSNYANWVQQKPGQAPRGLIGGTNKRAPGVPARFSGSLLGDKAALTLLGAQPEDEAEYYCALWASNLWVFGQGTKLTVL

SEQ ID NO: 92 - protein, 109 aa, Artificial
  synthetic
QAVVTQEPSLTVSPGGTVTLTCRSSTGAVTTSNYANWVQQKPGQAPRGLIGGTNKRAPGVPARFSGSLLGDKAALTLLGAQPEDEAEYYCALWYRNLWVFGQGTKLTVL

SEQ ID NO: 93 - protein, 109 aa, Artificial
  synthetic
QAVVTQEPSLTVSPGGTVTLTCRSSTGAVTTSNYANWVQQKPGQAPRGLIGGTNKRAPGVPARFSGSLLGDKAALTLLGAQPEDEAEYYCALWYSGLWVFGQGTKLTVL

SEQ ID NO: 94 - protein, 109 aa, Artificial
  synthetic
QAVVTQEPSLTVSPGGTVTLTCRSSTGAVGGSNYANWVQQKPGQAPRGLIGGTNKRAPGVPARFSGSLLGDKAALTLLGAQPEDEAEYYCALWYSNLWVFGQGTKLTVL

SEQ ID NO: 95 - protein, 109 aa, Artificial
  synthetic
QAVVTQEPSLTVSPGGTVTLTCRSSTGAVTTRGYANWVQQKPGQAPRGLIGGTNKRAPGVPARFSGSLLGDKAALTLLGAQPEDEAEYYCALWYSNLWVFGQGTKLTVL

SEQ ID NO: 96 - protein, 109 aa, Artificial
  synthetic
QAVVTQEPSLTVSPGGTVTLTCRSSTGAVTTSNYANWVQQKPGQAPRGLIGGTNKRAPGVPARFSGSLLGDKAALTLLGAQPEDEAEYYCALAASNLWVFGQGTKLTVL

SEQ ID NO: 97 - protein, 109 aa, Artificial
  synthetic
QAVVTQEPSLTVSPGGTVTLTCRSSTGAVTTSNYANWVQQKPGQAPRGLIGGTNKRAPGVPARFSGSLLGDKAALTLLGAQPEDEAEYYCALWYRGLWVFGQGTKLTVL

SEQ ID NO: 98 - protein, 109 aa, Artificial
  synthetic
QAVVTQEPSLTVSPGGTVTLTCRSSTGAVTTSNYANWVQQKPGQAPRGLIGGTNSRAPGVPARFSGSLLGDKAALTLLGAQPEDEAEYYCALWYSNLWVFGQGTKLTVL

SEQ ID NO: 99 - protein, 109 aa, Artificial
  synthetic
QAVVTQEPSLTVSPGGTVTLTCRSSTGAVTTSNYANWVQQKPGQAPRGLIGGTNSRAPGVPARFSGSLLGDKAALTLLGAQPEDEAEYYCALWYSDLWVFGQGTKLTVL

SEQ ID NO: 100 - protein, 330 aa, Artificial
  synthetic
ASTKGPSVFPLAPSSKSTSGGTAALGCLVKDYFPEPVTVSWNSGALTSGVHTFPAVLQSSGLYSLSSVVTVPSSSLGTQTYICNVNHKPSNTKVDKKVEPKSCDKTHTCPPCPAPEAAGGPSVFLFPPKPKDTLMISRTPEVTCVVVDVSHEDPEVKFNWYVDGVEVHNAKTKPREEQYNSTYRVVSVLTVLHQDWLNGKEYKCKVSNKALPAPIEKTISKAKGQPREPQVYTLPPSREEMTKNQVSLTCLVKGFYPSDIAVEWESNGQPENNYKTTPPVLDSDGSFFLYSKLTVDKSRWQQGNVFSCSVMHEALHNHYTQKSLSLSPGK

SEQ ID NO: 101 - protein, 106 aa, Artificial
  synthetic
GQPKAAPSVTLFPPSSEELQANKATLVCLISDFYPGAVTVAWKADSSPVKAGVETTTPSKQSNNKYAASSYLSLTPEQWKSHRSYSCQVTHEGSTVEKTVAPTECS

SEQ ID NO: 102 - protein, 107 aa, Artificial [sequence omitted]

SEQ ID NO: 103 - protein, 10 aa, Artificial
  synthetic
  misc_feature (5): Xaa is selected from N, G, S, D or E，preferably  N, G or S
  misc_feature (6): Xaa is selected from T, G, L or R，preferably  T or G
  misc_feature (7): Xaa is selected from Y, G, A or S，preferably  Y, A or S
GFTFXXXAMN

SEQ ID NO: 104 - protein, 19 aa, Artificial
  synthetic
  misc_feature (3): Xaa is selected from R, G, A or S，preferably  R or S
  misc_feature (4): Xaa is selected from S, G, L or R，preferably  S or L
  misc_feature (6): Xaa is selected from Y, G, A or S，preferably  Y or A
  misc_feature (7): Xaa is selected from N, G, S, D or E，preferably  N or G
  misc_feature (8): Xaa is selected from N, G, S, D or E，preferably  N or G
RIXXKXXXYATYYADSVKD

SEQ ID NO: 105 - protein, 14 aa, Artificial
  synthetic
  misc_feature (1): Xaa is selected from H, G, A or S，preferably  H or A
  misc_feature (2): Xaa is G or Y
  misc_feature (3): Xaa is selected from N, G, S, D or E，preferably  N or G
  misc_feature (4): Xaa is selected from F, G, A or S，preferably  F or A
  misc_feature (5): Xaa is G or Y
  misc_feature (6): Xaa is selected from N, G, S, D or E，preferably  N, Q or G
  misc_feature (7): Xaa is selected from S, G, L or R，preferably  S or R
  misc_feature (8): Xaa is selected from Y, G, A or S，preferably  Y or A
  misc_feature (9): Xaa is selected from V or A
XXXXXXXXXSWFAY

SEQ ID NO: 106 - protein, 13 aa, Artificial
  synthetic
  misc_feature (1)..(1): Xaa is selected from R, G, A or S，preferably  R or G
  misc_feature (8): Xaa is selected from T, G, L or R，preferably  T or G
  misc_feature (9): Xaa is selected from T, G, L or R，preferably  T or G
  misc_feature (10): Xaa is selected from S, G, L or R，preferably  S or R
XSSTGAVXXXYAN

SEQ ID NO: 107 - protein, 9 aa, Artificial
  synthetic
  misc_feature (3): Xaa is selected from W, G, A or S，preferably  W or A
  misc_feature (4): Xaa is selected from Y, G, A or S，preferably  Y or A
  misc_feature (5): Xaa is selected from S, G, L or R，preferably  S or R
  misc_feature (6): Xaa is selected from N, G, S, D or E，preferably  N, G or D
ALXXXXLWV

SEQ ID NO: 108 - protein, 100 aa, Artificial
  synthetic
EVQLVESGGGLVQPGGSLKLSCAASGFTFSGSAMHWVRQASGKGLEWVGRIRSKANSYATAYAASVKGRFTISRDDSKNTAYLQMNSLKTEDTAVYYCTR

SEQ ID NO: 109 - protein, 96 aa, Artificial
  synthetic
EIVMTQSPPTLSLSPGERVTLSCRASQSVSSSYLSWYQQKPGQAPRLLIYGASTRATGIPARFSGSGSGTDFTLTISSLQPEDFAVYYCQQDYNLP

SEQ ID NO: 110 - protein, 98 aa, Artificial
  synthetic
QAVVTQEPSLTVSPGGTVTLTCGSSTGAVTSGHYPYWFQQKPGQAPRTLIYDTSNKHSWTPARFSGSLLGGKAALTLLGAQPEDEAEYYCLLSYSGAR

SEQ ID NO: 111 - protein, 11 aa, Artificial
  synthetic
WGQGTTVTVSS

SEQ ID NO: 112 - protein, 10 aa, Artificial
  synthetic
FGQGTKVEIK

SEQ ID NO: 113 - protein, 10 aa, Artificial
  synthetic
FGGGTKLTVL

SEQ ID NO: 114 - protein, 118 aa, Artificial
  synthetic
EVQLVESGGGLVQPGGSLRLSCAASGFNIKDTYIHWVRQAPGKGLEWVARIYPTNGYTRYADSVKGRFTISADTSKNTAYLQMNSLRAEDTAVYYCSRWGGDGFYAMDYWGQGTLVTV

SEQ ID NO: 115 - protein, 107 aa, Artificial [sequence omitted]

SEQ ID NO: 116 - protein, 107 aa, Artificial [sequence omitted]

SEQ ID NO: 117 - protein, 330 aa, Artificial
  synthetic
ASTKGPSVFPLAPSSKSTSGGTAALGCLVKDYFPEPVTVSWNSGALTSGVHTFPAVLQSSGLYSLSSVVTVPSSSLGTQTYICNVNHKPSNTKVDKKVEPKSCDKTHTCPPCPAPEAAGGPSVFLFPPKPKDTLMISRTPEVTCVVVDVSHEDPEVKFNWYVDGVEVHNAKTKPREEQYNSTYRVVSVLTVLHQDWLNGKEYKCKVSNKALPAPIEKTISKAKGQPREPQVYTLPPSRDELTKNQVSLWCLVKGFYPSDIAVEWESNGQPENNYKTTPPVLDSDGSFFLYSKLTVDKSRWQQGNVFSCSVMHEALHNHYTQKSLSLSPGK

SEQ ID NO: 118 - protein, 330 aa, Artificial
  synthetic
ASTKGPSVFPLAPSSKSTSGGTAALGCLVKDYFPEPVTVSWNSGALTSGVHTFPAVLQSSGLYSLSSVVTVPSSSLGTQTYICNVNHKPSNTKVDKKVEPKSCDKTHTCPPCPAPEAAGGPSVFLFPPKPKDTLMISRTPEVTCVVVDVSHEDPEVKFNWYVDGVEVHNAKTKPREEQYNSTYRVVSVLTVLHQDWLNGKEYKCKVSNKALPAPIEKTISKAKGQPREPQVYTLPPSRDELTKNQVSLSCAVKGFYPSDIAVEWESNGQPENNYKTTPPVLDSDGSFFLVSKLTVDKSRWQQGNVFSCSVMHEALHNHYTQKSLSLSPGK

SEQ ID NO: 119 - protein, 330 aa, Artificial
  synthetic
ASTKGPSVFPLAPSSKSTSGGTAALGCLVKDYFPEPVTVSWNSGALTSGVHTFPAVLQSSGLYSLSSVVTVPSSSLGTQTYICNVNHKPSNTKVDKKVEPKSCDKTHTCPPCPAPEAAGGPSVFLFPPKPKDTLMISRTPEVTCVVVDVSHEDPEVKFNWYVDGVEVHNAKTKPREEQYNSTYRVVSVLTVLHQDWLNGKEYKCKVSNKALPAPIEKTISKAKGQPREPQVYTLPPCRDELTKNQVSLWCLVKGFYPSDIAVEWESNGQPENNYKTTPPVLDSDGSFFLYSKLTVDKSRWQQGNVFSCSVMHEALHNHYTQKSLSLSPGK

SEQ ID NO: 120 - protein, 330 aa, Artificial
  synthetic
ASTKGPSVFPLAPSSKSTSGGTAALGCLVKDYFPEPVTVSWNSGALTSGVHTFPAVLQSSGLYSLSSVVTVPSSSLGTQTYICNVNHKPSNTKVDKKVEPKSCDKTHTCPPCPAPEAAGGPSVFLFPPKPKDTLMISRTPEVTCVVVDVSHEDPEVKFNWYVDGVEVHNAKTKPREEQYNSTYRVVSVLTVLHQDWLNGKEYKCKVSNKALPAPIEKTISKAKGQPREPQVCTLPPSRDELTKNQVSLSCAVKGFYPSDIAVEWESNGQPENNYKTTPPVLDSDGSFFLVSKLTVDKSRWQQGNVFSCSVMHEALHNHYTQKSLSLSPGK

SEQ ID NO: 121 - protein, 452 aa, Artificial
  synthetic
EVQLLDSGGGLVQPGGSLRLSCAASGFTFSSYVMSWVRQAPGKGLNWVSTISHSGGSTYYADSVKGRFTISRDNSKNTLYLQMNSLRAEDTAVYYCAIDAPYYDILTGYRYWGQGTLVTVSSASTKGPSVFPLAPSSKSTSGGTAALGCLVKDYFPEPVTVSWNSGALTSGVHTFPAVLQSSGLYSLSSVVTVPSSSLGTQTYICNVNHKPSNTKVDKKVEPKSCDKTHTCPPCPAPEAAGGPSVFLFPPKPKDTLMISRTPEVTCVVVDVSHEDPEVKFNWYVDGVEVHNAKTKPREEQYNSTYRVVSVLTVLHQDWLNGKEYKCKVSNKALPAPIEKTISKAKGQPREPQVYTLPPSRDELTKNQVSLWCLVKGFYPSDIAVEWESNGQPENNYKTTPPVLDSDGSFFLYSKLTVDKSRWQQGNVFSCSVMHEALHNHYTQKSLSLSPGK

SEQ ID NO: 122 - protein, 214 aa, Artificial
  synthetic
DIQMTQSPSTLSASVGDRVTITCRASQSISSWLAWYQQKPGKAPKLLIYKASSLESGVPSRFSGSGSGTEFTLTISSLQPDDFATYYCQQYNSYSYTFGQGTKLEIKRTVAAPSVFIFPPSDEQLKSGTASVVCLLNNFYPREAKVQWKVDNALQSGNSQESVTEQDSKDSTYSLSSTLTLSKADYEKHKVYACEVTHQGLSSPVTKSFNRGEC

SEQ ID NO: 123 - protein, 455 aa, Artificial
  synthetic
EVQLVESGGGLVQPGGSLKLSCAASGFTFNTYAMNWVRQASGKGLEWVGRIRSKYNNYATYYADSVKDRFTISRDDSKSTLYLQMNSLKTEDTAVYYCARHGNFGQSYVSWFAYWGQGTTVTVSSASTKGPSVFPLAPSSKSTSGGTAALGCLVKDYFPEPVTVSWNSGALTSGVHTFPAVLQSSGLYSLSSVVTVPSSSLGTQTYICNVNHKPSNTKVDKKVEPKSCDKTHTCPPCPAPEAAGGPSVFLFPPKPKDTLMISRTPEVTCVVVDVSHEDPEVKFNWYVDGVEVHNAKTKPREEQYNSTYRVVSVLTVLHQDWLNGKEYKCKVSNKALPAPIEKTISKAKGQPREPQVYTLPPSRDELTKNQVSLSCAVKGFYPSDIAVEWESNGQPENNYKTTPPVLDSDGSFFLVSKLTVDKSRWQQGNVFSCSVMHEALHNHYTQKSLSLSPGK

SEQ ID NO: 124 - protein, 215 aa, Artificial
  synthetic
QAVVTQEPSLTVSPGGTVTLTCRSSTGAVTTSNYANWVQQKPGQAPRGLIGGTNKRAPGVPARFSGSLLGDKAALTLLGAQPEDEAEYYCALWYSNLWVFGQGTKLTVLGQPKAAPSVTLFPPSSEELQANKATLVCLISDFYPGAVTVAWKADSSPVKAGVETTTPSKQSNNKYAASSYLSLTPEQWKSHRSYSCQVTHEGSTVEKTVAPTECS

SEQ ID NO: 125 - protein, 455 aa, Artificial
  synthetic
EVQLVESGGGLVQPGGSLKLSCAASGFTFNTYAMNWVRQASGKGLEWVGRIRSKYNNYATYYADSVKDRFTISRDDSKSTLYLQMNSLKTEDTAVYYCARHYNFGQSYVSWFAYWGQGTTVTVSSASTKGPSVFPLAPSSKSTSGGTAALGCLVKDYFPEPVTVSWNSGALTSGVHTFPAVLQSSGLYSLSSVVTVPSSSLGTQTYICNVNHKPSNTKVDKKVEPKSCDKTHTCPPCPAPEAAGGPSVFLFPPKPKDTLMISRTPEVTCVVVDVSHEDPEVKFNWYVDGVEVHNAKTKPREEQYNSTYRVVSVLTVLHQDWLNGKEYKCKVSNKALPAPIEKTISKAKGQPREPQVYTLPPSRDELTKNQVSLSCAVKGFYPSDIAVEWESNGQPENNYKTTPPVLDSDGSFFLVSKLTVDKSRWQQGNVFSCSVMHEALHNHYTQKSLSLSPGK

SEQ ID NO: 126 - protein, 455 aa, Artificial
  synthetic
EVQLVESGGGLVQPGGSLKLSCAASGFTFNTYAMNWVRQASGKGLEWVGRIRSKAGGYATYYADSVKDRFTISRDDSKSTLYLQMNSLKTEDTAVYYCARHGNFGQSYVSWFAYWGQGTTVTVSSASTKGPSVFPLAPSSKSTSGGTAALGCLVKDYFPEPVTVSWNSGALTSGVHTFPAVLQSSGLYSLSSVVTVPSSSLGTQTYICNVNHKPSNTKVDKKVEPKSCDKTHTCPPCPAPEAAGGPSVFLFPPKPKDTLMISRTPEVTCVVVDVSHEDPEVKFNWYVDGVEVHNAKTKPREEQYNSTYRVVSVLTVLHQDWLNGKEYKCKVSNKALPAPIEKTISKAKGQPREPQVYTLPPSRDELTKNQVSLSCAVKGFYPSDIAVEWESNGQPENNYKTTPPVLDSDGSFFLVSKLTVDKSRWQQGNVFSCSVMHEALHNHYTQKSLSLSPGK